European Patent Specification EP 3 728 583 B1, published March 1, 2023. Title: COUNTER-SELECTION BY INHIBITION OF CONDITIONALLY ESSENTIAL GENES. Applicant: Novozymes A/S. The sequence listing filed with the application follows.

SEQUENCE LISTING (15 sequences)

SEQ ID NO: 1 - DNA, 4107 bp, Streptococcus pyogenes
atggacaaaaaatacagcatcggcctggatattggcacaaattcagttggctgggcagttatcacagacgaatataaagttccgagcaaaaaatttaaagtcctgggcaatacagatcgccatagcatcaaaaaaaacctgattggcgcactgctgtttgattcaggcgaaacagcagaagcaacaagacttaaaagaacagcaagacgcagatatacaagacgcaaaaatcgcatttgctatctgcaagaaatctttagcaacgaaatggcgaaagtcgacgacagcttttttcatagactggaagaatcatttctggtcgaagaagataaaaaacacgaacgccatccgatttttggcaacattgttgatgaagtcgcgtatcatgaaaaatacccgacaatttatcatctgcgcaaaaaactggttgacagcacagataaagcagatcttcgcctgatttatctggcactggcacatatgatcaaatttagaggccattttctgatcgaaggcgatctgaatccggataattcagatgtcgacaaactgtttattcagctggtccagacatataaccagctgtttgaagaaaatccgattaatgcatcaggcgttgatgcaaaagcaattctgtcagcaagactgtcaaaatcaagacgcctggaaaatctgattgcacaactgcctggcgaaaaaaaaaatggactgtttggcaatcttattgcactgtcactgggcctgacaccgaactttaaatcaaattttgatctggcggaagatgcgaaactgcaactttcaaaagatacgtatgatgacgatctggataatctgctggcgcaaattggcgatcaatatgcagatctttttctggcagcgaaaaatctgtcagatgcaattctgctgtcagatattctgcgcgtcaatacagaaattacaaaagcaccgctgagcgcgagcatgattaaaagatatgatgaacatcatcaggacctgacactgctgaaagcactggttagacaacaactgccggaaaaatacaaagaaatcttttttgatcagagcaaaaacggctatgcaggctatattgatggcggagcatcacaagaagaattttacaaatttatcaaaccgatcctggaaaaaatggatggaacagaagaactgctggttaaactgaatcgcgaagatttactgagaaaacagcgcacatttgataatggctcaattccgcatcaaattcatctgggcgaactgcatgcgattcttagacgccaagaagatttttatccgtttctgaaagacaaccgggaaaaaattgaaaaaatcctgacatttcgcatcccgtattatgtcggaccgctggcaagaggcaattcaagatttgcatggatgacacgcaaaagcgaagaaacaattacaccgtggaattttgaagaagtcgttgataaaggcgcaagcgcacaatcatttattgaacgcatgacgaactttgacaaaaacctgccgaatgaaaaagtcctgccgaaacattcactgctgtatgaatactttacggtctataatgaactgacgaaagtcaaatatgtcacagaaggcatgagaaaaccggcatttctgtcaggcgaacagaaaaaagcgattgtcgatcttctgtttaaaacgaaccgcaaagtcacagtgaaacagctgaaagaagattactttaaaaaaatcgaatgctttgatagcgtcgaaatctcaggcgtcgaagatagatttaatgcaagcctgggcacatatcatgatctgctgaaaatcatcaaagataaagattttctggataacgaagaaaacgaagatatcctggaagatattgtgctgacactgacgctttttgaagatcgcgaaatgattgaagaacgcctgaaaacatatgcgcacctgtttgatgataaagtcatgaaacaacttaaacgcagacgctatacaggctggggcagactttcaagaaaactgattaacggcattcgcgataaacaaagcggcaaaacaatcctggattttctgaaatcagatggctttgcgaatcgcaattttatgcagctgattcatgatgacagcctgacgtttaaagaagatattcagaaagcacaagtttcaggccaaggcgattcactgcatgaacatattgcaaatctggcaggctcaccggcaatcaaaaaaggcattctgcaaacagttaaagtcgtcgatgaactggttaaagttatgggcagacataaaccggaaaacatcgttattgaaatggcacgcgaaaatcagacaacacaaaaaggacagaaaaattcacgcgaacggatgaaaagaattgaagaaggcattaaagaactgggcagccaaatcctgaaagaacatccggttgaaaatacacagctgcagaacgaaaaactgtatctgtattatctgcagaatggacgcgatatgtatgtcgatcaagaactggatattaatcgcctgagcgattatgatgtggatcatattgttccgcagagctttcttaaagatgatagcatcgataacaaagtcctgacacgctcagataaaaacagaggcaaatcagataatgtcccgtcagaagaggttgtcaaaaaaatgaaaaactactggcgtcaactgctgaacgcgaaacttattacacaacgcaaatttgacaatctgacaaaagcagaaagaggcggactgtcagaacttgataaagcgggttttatcaaaagacagctggtcgaaacacgccagattacaaaacatgttgcgcaaattctggatagccgcatgaacacaaaatatgacgaaaacgataaactgatccgggaagtcaaagtcattacgctgaaatcaaaactggtcagcgattttcgcaaagactttcagttttacaaagtccgcgaaatcaacaactaccatcatgcacatgatgcatatctgaatgcagttgtcggcacagcgcttatcaaaaaataccctaaactggaaagcgaatttgtctacggcgactataaagtctatgatgtccgcaaaatgattgcgaaaagcgaacaagaaattggcaaagcgacagcgaaatactttttttacagcaacatcatgaacttttttaaaacggaaatcacactggcgaacggcgaaattagaaaaagaccgcttattgaaacgaacggtgaaacaggcgaaattgtttgggataaaggcagagattttgcaacagttagaaaagttctgagcatgccgcaagtcaacatcgtgaaaaaaacagaagttcagacaggcggatttagcaaagaatcaattcttccgaaacgcaactcagacaaactgattgcgcgtaaaaaagactgggacccgaaaaaatacggtggctttgattcaccgacagttgcatattcagttctggttgttgcgaaagtggaaaaaggcaaatccaaaaaacttaaaagcgtgaaagaacttctgggcatcacaattatggaacgctcgagctttgaaaaaaacccgatcgactttctggaagccaaaggctataaagaagtgaaaaaagaccttattatcaaactgccgaaatacagcctgtttgaactggaaaatggcagaaaacgcatgctggcatcagcaggcgaacttcagaaaggcaatgaactggcactgccgtcaaaatatgttaactttctgtatctggcgagccattacgaaaaacttaaaggctcaccggaagataacgaacagaaacaactgtttgtcgaacagcataaacattacctggacgaaatcatcgaacaaatcagcgaattttcaaaacgcgttattctggcagatgcgaacctggataaagttcttagcgcatataacaaacaccgggataaaccgattagagaacaagcggaaaatatcattcacctgtttacactgacaaatcttggcgcaccggcagcgtttaaatactttgatacaacaattgaccgcaaacgctacacaagcacaaaagaagttctggacgcaacactgattcatcaatcaattacaggcctttatgaaacgcgcattgatctgtcacaactgggaggcgattga

SEQ ID NO: 2 - protein, 1368 aa, Streptococcus pyogenes [sequence omitted]

SEQ ID NO: 3 - DNA, 5888 bp, Artificial Sequence
  Sequence of bglC-cas9d locus
tgtttttgataagatcacggagtttatccggaaaccgttcatgaagaagaagcagacgattgatgaacaagggcatgtagaaacgaaaaaagtgccgaaatcaaacttcggctatttgctgaattgctattggtgcgcagggatatggtgcgcgttgatcattgctgtcggatatctgattgccccaaaagcgatattcccgttgattttgattttgtcggtcgccggggggcaggcgattcttgaaacgtttgtcggtgtcgccacaaaacttgtcggctttttctccgatttaaagaagtaaaccattccaagcggatggttttatttttttgtcaataaagtgatacaaacagcagagagaacgtgtcagttttatgaacttttcacagcgatttttcccggatgcggcattttaggcagagaggaagcatctcattgtaaagatttcagtttttaaaatttagaattgagagaaaaaggatgtgcaaagtccccggagctcggatccactagtaacggccgccagtgtgctggaattcgcccttgcggccgctcgctttccaatctgaaggtttcattgtgggatgttgatccggaagattggaagtacaaaaataagcaaaagattgtcaatcatgtcatgagccatgcgggagacggaaaaatcgtcttaatgcacgatatttatgcaacgtccgcagatgctgctgaagagattattaaaaagctgaaagcaaaaggctatcaattggtaactgtatctcagcttgaagaagtgaagaagcagagaggctattgaataaatgagtagaaagcgccatatcggcgcttttcttttggaagaaaatatagggaaaatggtacttgttaaaaattcggaatatttatacaatatcatatgtatcacattgaaaggggaggagaatcatggacaaaaaatacagcatcggcctggctattggcacaaattcagttggctgggcagttatcacagacgaatataaagttccgagcaaaaaatttaaagtcctgggcaatacagatcgccatagcatcaaaaaaaacctgattggcgcactgctgtttgattcaggcgaaacagcagaagcaacaagacttaaaagaacagcaagacgcagatatacaagacgcaaaaatcgcatttgctatctgcaagaaatctttagcaacgaaatggcgaaagtcgacgacagcttttttcatagactggaagaatcatttctggtcgaagaagataaaaaacacgaacgccatccgatttttggcaacattgttgatgaagtcgcgtatcatgaaaaatacccgacaatttatcatctgcgcaaaaaactggttgacagcacagataaagcagatcttcgcctgatttatctggcactggcacatatgatcaaatttagaggccattttctgatcgaaggcgatctgaatccggataattcagatgtcgacaaactgtttattcagctggtccagacatataaccagctgtttgaagaaaatccgattaatgcatcaggcgttgatgcaaaagcaattctgtcagcaagactgtcaaaatcaagacgcctggaaaatctgattgcacaactgcctggcgaaaaaaaaaatggactgtttggcaatcttattgcactgtcactgggcctgacaccgaactttaaatcaaattttgatctggcggaagatgcgaaactgcaactttcaaaagatacgtatgatgacgatctggataatctgctggcgcaaattggcgatcaatatgcagatctttttctggcagcgaaaaatctgtcagatgcaattctgctgtcagatattctgcgcgtcaatacagaaattacaaaagcaccgctgagcgcgagcatgattaaaagatatgatgaacatcatcaggacctgacactgctgaaagcactggttagacaacaactgccggaaaaatacaaagaaatcttttttgatcagagcaaaaacggctatgcaggctatattgatggcggagcatcacaagaagaattttacaaatttatcaaaccgatcctggaaaaaatggatggaacagaagaactgctggttaaactgaatcgcgaagatttactgagaaaacagcgcacatttgataatggctcaattccgcatcaaattcatctgggcgaactgcatgcgattcttagacgccaagaagatttttatccgtttctgaaagacaaccgggaaaaaattgaaaaaatcctgacatttcgcatcccgtattatgtcggaccgctggcaagaggcaattcaagatttgcatggatgacacgcaaaagcgaagaaacaattacaccgtggaattttgaagaagtcgttgataaaggcgcaagcgcacaatcatttattgaacgcatgacgaactttgacaaaaacctgccgaatgaaaaagtcctgccgaaacattcactgctgtatgaatactttacggtctataatgaactgacgaaagtcaaatatgtcacagaaggcatgagaaaaccggcatttctgtcaggcgaacagaaaaaagcgattgtcgatcttctgtttaaaacgaaccgcaaagtcacagtgaaacagctgaaagaagattactttaaaaaaatcgaatgctttgatagcgtcgaaatctcaggcgtcgaagatagatttaatgcaagcctgggcacatatcatgatctgctgaaaatcatcaaagataaagattttctggataacgaagaaaacgaagatatcctggaagatattgtgctgacactgacgctttttgaagatcgcgaaatgattgaagaacgcctgaaaacatatgcgcacctgtttgatgataaagtcatgaaacaacttaaacgcagacgctatacaggctggggcagactttcaagaaaactgattaacggcattcgcgataaacaaagcggcaaaacaatcctggattttctgaaatcagatggctttgcgaatcgcaattttatgcagctgattcatgatgacagcctgacgtttaaagaagatattcagaaagcacaagtttcaggccaaggcgattcactgcatgaacatattgcaaatctggcaggctcaccggcaatcaaaaaaggcattctgcaaacagttaaagtcgtcgatgaactggttaaagttatgggcagacataaaccggaaaacatcgttattgaaatggcacgcgaaaatcagacaacacaaaaaggacagaaaaattcacgcgaacggatgaaaagaattgaagaaggcattaaagaactgggcagccaaatcctgaaagaacatccggttgaaaatacacagctgcagaacgaaaaactgtatctgtattatctgcagaatggacgcgatatgtatgtcgatcaagaactggatattaatcgcctgagcgattatgatgtggatgctattgttccgcagagctttcttaaagatgatagcatcgataacaaagtcctgacacgctcagataaaaacagaggcaaatcagataatgtcccgtcagaagaggttgtcaaaaaaatgaaaaactactggcgtcaactgctgaacgcgaaacttattacacaacgcaaatttgacaatctgacaaaagcagaaagaggcggactgtcagaacttgataaagcgggttttatcaaaagacagctggtcgaaacacgccagattacaaaacatgttgcgcaaattctggatagccgcatgaacacaaaatatgacgaaaacgataaactgatccgggaagtcaaagtcattacgctgaaatcaaaactggtcagcgattttcgcaaagactttcagttttacaaagtccgcgaaatcaacaactaccatcatgcacatgatgcatatctgaatgcagttgtcggcacagcgcttatcaaaaaataccctaaactggaaagcgaatttgtctacggcgactataaagtctatgatgtccgcaaaatgattgcgaaaagcgaacaagaaattggcaaagcgacagcgaaatactttttttacagcaacatcatgaacttttttaaaacggaaatcacactggcgaacggcgaaattagaaaaagaccgcttattgaaacgaacggtgaaacaggcgaaattgtttgggataaaggcagagattttgcaacagttagaaaagttctgagcatgccgcaagtcaacatcgtgaaaaaaacagaagttcagacaggcggatttagcaaagaatcaattcttccgaaacgcaactcagacaaactgattgcgcgtaaaaaagactgggacccgaaaaaatacggtggctttgattcaccgacagttgcatattcagttctggttgttgcgaaagtggaaaaaggcaaatccaaaaaacttaaaagcgtgaaagaacttctgggcatcacaattatggaacgctcgagctttgaaaaaaacccgatcgactttctggaagccaaaggctataaagaagtgaaaaaagaccttattatcaaactgccgaaatacagcctgtttgaactggaaaatggcagaaaacgcatgctggcatcagcaggcgaacttcagaaaggcaatgaactggcactgccgtcaaaatatgttaactttctgtatctggcgagccattacgaaaaacttaaaggctcaccggaagataacgaacagaaacaactgtttgtcgaacagcataaacattacctggacgaaatcatcgaacaaatcagcgaattttcaaaacgcgttattctggcagatgcgaacctggataaagttcttagcgcatataacaaacaccgggataaaccgattagagaacaagcggaaaatatcattcacctgtttacactgacaaatcttggcgcaccggcagcgtttaaatactttgatacaacaattgaccgcaaacgctacacaagcacaaaagaagttctggacgcaacactgattcatcaatcaattacaggcctttatgaaacgcgcattgatctgtcacaactgggaggcgattgaattgacactaaagggatccagaagcggcaacacgctaatcaataaaaaaacgctgtgcggttaaagggcacagcgtttttttgtgtatgaatcgaaaaagagaacagatcgcaggtctcaaaaatcgagcgtaaagggctgatccgcggccgcgtcgactagaagagcagagaggacggatttcctgaaggaaatccgtttttttattttgcccgtcttataaatttcgttgtccaactcgcttaattgcgagtttttatttcgtttatttcaatcaaggtaaatgctagcggccgcgtcgactagaagagcagagaggacggatttcctgaaggaaatccgtttttttattttgcccgtcttataaatttcgttgccatgggatccgcggccgcgctgcagccaacacgatagcagtacaatacagagcgggggacaacaatgtaaacggcaaccaaatccgccctcagctcaacattaaaaacaacagcaaaaaaaccgtctctttaaatcgaatcaccgtccgctactggtataaaacgaatcgcaaaggaaaaaattttgactgcgactatgcccaaatcggctgcagcaaaatcacgcacaaattcgtccaattaaaaaaagcggtaaacggagcagacacgtatcttgaagtagggtttaaaaatggtacattggcgccgggtgcaagtacaggtgaaatccagatccgtcttcacaatgacggctggagcaattatgcccaaagcggcgactattcatttttaaattcaaacacgtttaaaaatacgaaaaaaatcacgttgtatgagaacggaaagctgatttggggcactgaacctaaataa

SEQ ID NO: 4 - DNA, 3133 bp, Artificial Sequence
  Sequence of gnt locus of PP3811-gDNA3: gnt-dsRED-gDNA(cat)
agcgaagccttgtgcataggcgcagattttgcccatatataatgcctgtctgacgcggtcgatccacacgttttgatccaggcgccgttcttctgttgcaggtccggccaatactttttccgcagctgtccgttcgtcttttaatgatgacaggtaacgggcaaacagggattccgtgataattgatgatggaatgccgttgtcgacggcctgcaggctcgtccatttgcccgtgcctttttggccggttttgtcgaggatgacgtcgatgagtggagcgcccgtcttctcatcctttttccgcaggatctccgccgtgatttcgattaaatagctgttcagctctccttgattccacgtgtcgaaaatgtcagcgatttcatctatcggcaaaagaagcttttctcttaaaaacgtatatgcttcggcgatgagctgcatgtctgcgtattcgatgccgttgtgcaccattttgacaaaatgacccgcgcctttcggacggccgctcgctttccaatctgaaggtttcattgtgggatgttgatccggaagattggaagtacaaaaataagcaaaagattgtcaatcatgtcatgagccatgcgggagacggaaaaatcgtcttaatgcacgatatttatgcaacgtccgcagatgctgctgaagagattattaaaaagctgaaagcaaaaggctatcaattggtaactgtatctcagcttgaagaagtgaagaagcagagaggctattgaataaatgagtagaaagcgccatatcggcgcttttcttttggaagaaaatatagggaaaatggtacttgttaaaaattcggaatatttatacaatatcatatgtatcacattgaaaggaggggcctgctgtccagactgtccgctgtgtaaaaaaaaggaataaaggggggttgacattattttactgatatgtataatataatttgtataagaaaatggaggggccctcgaaacgtaagatgaaaccttagataaaagtgctttttttgttgcaattgaagaattattaatgttaagcttaattaaagataatatctttgaattgtaacgcccctcaaaagtaagaactacaaaaaaagaatacgttatatagaaatatgtttgaaccttcttcagattacaaatatattcggacggactctacctcaaatgcttatctaactatagaatgacatacaagcacaaccttgaaaatttgaaaatataactaccaatgaacttgttcatgtgaattatcgctgtatttaattttctcaattcaatatataatatgccaatacattgttacaagtagaaattaagacacccttgatagccttactatacctaacatgatgtagtattaaatgaatatgtaaatatatttatgataagaagcgacttatttataatcattacatatttttctattggaatgattaagattccaatagaatagtgtataaattatttatcttgaaaggagggatgcctaaaaacgaagaacattaaaaacatatatttgcaccgtctaatggatttatgaaaaatcattttatcagtttgaaaattatgtattatggagctctataaaaatgaggagggaaccgaatggcttcaactgaagacgtaatcaaagagttcatgcgcttcaaagtgcgaatggaaggaagtgtaaacgggcatgagtttgaaattgaaggtgaaggtgaaggaaggccttatgaaggaacgcaaactgcaaaacttaaagtgacaaaaggaggaccgctgccgtttgcttgggacatcttaagtccgcagtttcagtatgggtcaaaagtttatgtaaagcatcctgctgacattcctgattacaaaaagttaagttttcctgaaggattcaagtgggagcgcgtaatgaactttgaagatggaggtgtcgtaactgtaacgcaagattcaagtctgcaagacggttgcttcatttacaaagtaaagttcattggcgtgaactttccaagtgatggtcctgtaatgcagaaaaagacaatgggttgggagccgtcaactgagaggctttatccgcgtgatggtgtcttgaaaggtgaaattcacaaagccttaaagttgaaagatggagggcattatcttgttgagttcaagagcatttacatggcgaaaaagcctgtgcagcttcctggctactactatgttgattcaaaacttgacataactagtcacaacgaagactacacaattgttgagcagtatgagcgaactgaaggaaggcatcatctttttctttaatgctgtccagactgtccgctgtgtaaaaaaaaggaataaaggggggttgacattattttactgatatgtataatataatttgtataagaaaatgcttcatgtaatggtcaaaatgttttagagctagaaatagcaagttaaaataaggctagtccgttatcaacttgaaaaagtggcaccgagtcggtgctttctgataattgccaacacaattaacatctcaatcaaggtaaatgctagcggccgcgtcgactagaagagcagagaggacggatttcctgaaggaaatccgtttttttattttgcccgtcttataaatttcgttgagatcttttatacaaataggcttaacaataaagtaaatcctaatccggccaccgcgataattgtttcaagcagtgtccaggtggcgaatgtttctttcatgctcaggccgaaatactctttgaacatccagaagcccgcgtcgttgacatgggaagcgattacacttccggcccctgttgcaagcacaaccagtgcaagattgacatcgctttgtccgagcatcggaagaacgagtccggtcgtgcttaatgcagcaactgtcgcggaacctaaagagatgcgcagaatcgcggcgatgacccaggcgagcaagatcggcgacatggccgttcctttgaataattcagctacatagtcgcctactccgccgttgatcaagacttgtttgaatgcgccgccgcccccgatgatcaagagcatcattccgatttgagtaatggcggttgaacaggaatccatcacttgtttgatcgggatctttctggcgatacccatcgtataaatcg

SEQ ID NO: 5 - DNA, 2813 bp, Artificial Sequence
  Sequence of amyL locus in of PP3811-gDNA3: amyL-dsRED-gDNA(cat)
tacagaagcatgaagggcatgcgaccttctttgtgcttggaagcagagcgcaatattatcccgaaacgataaaacggatgctgaaggaaggaaacgaagtcggcaaccattcctgggaccatccgttattgacaaggctgtcaaacgaaaaagcgtatcaggagattaacgacacgcaagaaatgatcgaaaaaatcagcggacacctgcctgtacacttgcgtcctccatacggcgggatcaatgattccgtccgctcgctttccaatctgaaggtttcattgtgggatgttgatccggaagattggaagtacaaaaataagcaaaagattgtcaatcatgtcatgagccatgcgggagacggaaaaatcgtcttaatgcacgatatttatgcaacgtccgcagatgctgctgaagagattattaaaaagctgaaagcaaaaggctatcaattggtaactgtatctcagcttgaagaagtgaagaagcagagaggctattgaataaatgagtagaaagcgccatatcggcgcttttcttttggaagaaaatatagggaaaatggtacttgttaaaaattcggaatatttatacaatatcatatgtatcacattgaaaggaggggcctgctgtccagactgtccgctgtgtaaaaaaaaggaataaaggggggttgacattattttactgatatgtataatataatttgtataagaaaatggaggggccctcgaaacgtaagatgaaaccttagataaaagtgctttttttgttgcaattgaagaattattaatgttaagcttaattaaagataatatctttgaattgtaacgcccctcaaaagtaagaactacaaaaaaagaatacgttatatagaaatatgtttgaaccttcttcagattacaaatatattcggacggactctacctcaaatgcttatctaactatagaatgacatacaagcacaaccttgaaaatttgaaaatataactaccaatgaacttgttcatgtgaattatcgctgtatttaattttctcaattcaatatataatatgccaatacattgttacaagtagaaattaagacacccttgatagccttactatacctaacatgatgtagtattaaatgaatatgtaaatatatttatgataagaagcgacttatttataatcattacatatttttctattggaatgattaagattccaatagaatagtgtataaattatttatcttgaaaggagggatgcctaaaaacgaagaacattaaaaacatatatttgcaccgtctaatggatttatgaaaaatcattttatcagtttgaaaattatgtattatggagctcttataaaaatgaggagggaaccgaatggcttcaactgaagacgtaatcaaagagttcatgcgcttcaaagtgcgaatggaaggaagtgtaaacgggcatgagtttgaaattgaaggtgaaggtgaaggaaggccttatgaaggaacgcaaactgcaaaacttaaagtgacaaaaggaggaccgctgccgtttgcttgggacatcttaagtccgcagtttcagtatgggtcaaaagtttatgtaaagcatcctgctgacattcctgattacaaaaagttaagttttcctgaaggattcaagtgggagcgcgtaatgaactttgaagatggaggtgtcgtaactgtaacgcaagattcaagtctgcaagacggttgcttcatttacaaagtaaagttcattggcgtgaactttccaagtgatggtcctgtaatgcagaaaaagacaatgggttgggagccgtcaactgagaggctttatccgcgtgatggtgtcttgaaaggtgaaattcacaaagccttaaagttgaaagatggagggcattatcttgttgagttcaagagcatttacatggcgaaaaagcctgtgcagcttcctggctactactatgttgattcaaaacttgacataactagtcacaacgaagactacacaattgttgagcagtatgagcgaactgaaggaaggcatcatctttttctttaatgctgtccagactgtccgctgtgtaaaaaaaaggaataaaggggggttgacattattttactgatatgtataatataatttgtataagaaaatgcttcatgtaatggtcaaaatgttttagagctagaaatagcaagttaaaataaggctagtccgttatcaacttgaaaaagtggcaccgagtcggtgctttactgataattgccaacacaattaacatctcaatcaaggtaaatgctagcgcggccgcgtcgacaggcctctttgattacattttataattaattttaacaaagtgtcatcagccctcaggaaggacttgctgacagtttgaatcgcataggtaaggcggggatgaaatggcaacgttatctgatgtagcaaagaaagcaaatgtgtcgaaaatgacggtatcgcgggtgatcaatcatcctgagactgtgacggatgaattgaaaaagcttgttcattccgcaatgaaggagctcaattatataccgaactatgcagcaagagcgctcgttcaaaacagaacacaggtcgtcaagctgctcatactggaagaaatggatacaacagaaccttattatatgaatctgttaacgggaatcagccgcgagctggaccgtcatcattatgctttgcagcttgtcacaaggaaatctctcaatatcggccagtgcgacggcattattgcgacggggttgagaaaagccgattttgaagggctcatcaaggtttttgaaaagcctgtcgttgta

SEQ ID NO: 6 - DNA, 3045 bp, Artificial Sequence
  Sequence of lacA2 locus in of PP3811-gDNA3: lacA2-dsRED-gDNA(cat)
tgttgattggctttggcctccagctttttataaatggattcaccgaagctggttaagtagatatagtggttgcggctgtcctcctcgcttctctttttatagaccatattttctttttcaaaccgcttcaggatccggctgacatagccccggtccaggccgagcgtatcttgaatcagtttggctgtacaatcggccgtattgtgaatttcaaataatatccgggtttccgtcaatgaaaaagggctgtcataaatatgttcattcagaaaaccgagcacatttgtatagaatcgattgaactttctgaattttaaagtgatagaatgattgatttctgtcatctcaaaacctctctccctgtaaatcgttgctttaatcaattataataaaatagttgatttagtcaagtgtatggaaatgaagttaaaaatgttaatgatagattatattttacaaataaagaaagataaattcaatcatacaggaaaattcatccagcggccgctcgctttccaatctgaaggtttcattgtgggatgttgatccggaagattggaagtacaaaaataagcaaaagattgtcaatcatgtcatgagccatgcgggagacggaaaaatcgtcttaatgcacgatatttatgcaacgtccgcagatgctgctgaagagattattaaaaagctgaaagcaaaaggctatcaattggtaactgtatctcagcttgaagaagtgaagaagcagagaggctattgaataaatgagtagaaagcgccatatcggcgcttttcttttggaagaaaatatagggaaaatggtacttgttaaaaattcggaatatttatacaatatcatatgtatcacattgaaaggaggggcctgctgtccagactgtccgctgtgtaaaaaaaaggaataaaggggggttgacattattttactgatatgtataatataatttgtataagaaaatggaggggccctcgaaacgtaagatgaaaccttagataaaagtgctttttttgttgcaattgaagaattattaatgttaagcttaattaaagataatatctttgaattgtaacgcccctcaaaagtaagaactacaaaaaaagaatacgttatatagaaatatgtttgaaccttcttcagattacaaatatattcggacggactctacctcaaatgcttatctaactatagaatgacatacaagcacaaccttgaaaatttgaaaatataactaccaatgaacttgttcatgtgaattatcgctgtatttaattttctcaattcaatatataatatgccaatacattgttacaagtagaaattaagacacccttgatagccttactatacctaacatgatgtagtattaaatgaatatgtaaatatatttatgataagaagcgacttatttataatcattacatatttttctattggaatgattaagattccaatagaatagtgtataaattatttatcttgaaaggagggatggctaaaaacgaagaacattaaaaacatatatttgcaccgtctaatggatttatgaaaaatcattttatcagtttgaaaattatgtattatggagctctataaaaatgaggagggaaccgaatggcatctacagaagatgtgatcaaggaattcatgcggtttaaggtgagaatggaaggaagcgtgaacggacatgaatttgaaatcgagggggaaggcgaaggcagaccctatgaaggtacacagacagcaaagctgaaggtgacaaagggtggaccgctgccttttgcctgggacatcctgagcccacagtttcaatatgggagtaaggtgtacgtgaagcatccggctgacatcccggactataagaagctgtccttcccagagggctttaagtgggaaagagtcatgaatttcgaagatggcggtgtggtgacagtgacgcaagatagctccctgcaagatggatgctttatctacaaggtgaagttcatcggagtgaatttcccttcggatggaccggtgatgcaaaagaagacaatgggatgggaacctagtacagaaaggctgtatccgagagatggagtgctgaagggagaaatccacaaggcgctgaagctgaaggatggcggacactatctggtggagtttaagagcatctatatggccaagaagccagtgcaactgcctgggtactactatgtggactcgaagctggatatcacttcacataacgaagactacacaatcgtggaacaatatgaacggacggaaggaaggcatcacctgtttctgtaatgctgtccagactgtccgctgtgtaaaaaaaaggaataaaggggggttgacattattttactgatatgtataatataatttgtataagaaaatgcttcatgtaatggtcaaaatgttttagagctagaaatagcaagttaaaataaggctagtccgttatcaacttgaaaaagtggcaccgagtcggtgctttctgataattgccaacacaattaacatctcaatcaaggtaaatgctagcatcgattacaacccggatcaatggcttaaatatccggacgtattaaaagaagatatccgcctgatgaaactgtcccgctgcaatgtgatgtctgtcggcattttctcctgggtttcgctcgagcctgaagaaggaagatttacatttgactggctcgatcaggttcttgatactttcaaggaaaacggaatttatgcgtttttggctacaccgagcggtgccagaccggcttggatgtccaaaaagtatccagaggtgctgagaacggagcgcaacagggtcagaaaccttcacggaaagcggcacaatcactgctatacgtcgcctgtctaccgccggaaaacggcgatcataaacggaaagctcgcggagcgctatgcgcatcacccggccgtcatcggctggcacatttctaatgaatacggcggagaatgccattgtgaactttgccaagacaagttcagagagtggctgctggcgaaatacaaaacgctggaccgcc

SEQ ID NO: 7 - DNA, 3915 bp, Artificial Sequence
  Sequence of the gnt locus after integration of amyL in PP3811-amyL3
agcgaagccttgtgcataggcgcagattttgcccatatataatgcctgtctgacgcggtcgatccacacgttttgatccaggcgccgttcttctgttgcaggtccggccaatactttttccgcagctgtccgttcgtcttttaatgatgacaggtaacgggcaaacagggattccgtgataattgatgatggaatgccgttgtcgacggcctgcaggctcgtccatttgcccgtgcctttttggccggttttgtcgaggatgacgtcgatgagtggagcgcccgtcttctcatcctttttccgcaggatctccgccgtgatttcgattaaatagctgttcagctctccttgattccacgtgtcgaaaatgtcagcgatttcatctatcggcaaaagaagcttttctcttaaaaacgtatatgcttcggcgatgagctgcatgtctgcgtattcgatgccgttgtgcaccattttgacaaaatgacccgcgcctttcggacggccgctcgctttccaatctgaaggtttcattgtgggatgttgatccggaagattggaagtacaaaaataagcaaaagattgtcaatcatgtcatgagccatgcgggagacggaaaaatcgtcttaatgcacgatatttatgcaacgtccgcagatgctgctgaagagattattaaaaagctgaaagcaaaaggctatcaattggtaactgtatctcagcttgaagaagtgaagaagcagagaggctattgaataaatgagtagaaagcgccatatcggcgcttttcttttggaagaaaatatagggaaaatggtacttgttaaaaattcggaatatttatacaatatcatatgtatcacattgaaaggaggggcctgctgtccagactgtccgctgtgtaaaaaaaaggaataaaggggggttgacattattttactgatatgtataatataatttgtataagaaaatggaggggccctcgaaacgtaagatgaaaccttagataaaagtgctttttttgttgcaattgaagaattattaatgttaagcttaattaaagataatatctttgaattgtaacgcccctcaaaagtaagaactacaaaaaaagaatacgttatatagaaatatgtttgaaccttcttcagattacaaatatattcggacggactctacctcaaatgcttatctaactatagaatgacatacaagcacaaccttgaaaatttgaaaatataactaccaatgaacttgttcatgtgaattatcgctgtatttaattttctcaattcaatatataatatgccaatacattgttacaagtagaaattaagacacccttgatagccttactatacctaacatgatgtagtattaaatgaatatgtaaatatatttatgataagaagcgacttatttataatcattacatatttttctattggaatgattaagattccaatagaatagtgtataaattatttatcttgaaaggagggatgcctaaaaacgaagaacattaaaaacatatatttgcaccgtctaatggatttatgaaaaatcattttatcagtttgaaaattatgtattatggccacattgaaaggggaggagaatcatgaaacaacaaaaacggctttacgcccgattgctgacgctgttatttgcgctcatcttcttgctgcctcattctgcagcagcggcggcaaatcttaatgggacgctgatgcagtattttgaatggtacatgcccaatgacggccaacattggaggcgtttgcaaaacgactcggcatatttggctgaacacggtattactgccgtctggattcccccggcatataagggaacgagccaagcggatgtgggctacggtgcttacgacctttatgatttaggggagtttcatcaaaaagggacggttcggacaaagtacggcacaaaaggagagctgcaatctgcgatcaaaagtcttcattcccgcgacattaacgtttacggggatgtggtcatcaaccacaaaggcggcgctgatgcgaccgaagatgtaaccgcggttgaagtcgatcccgctgaccgcaaccgcgtaatttcaggagaacacctaattaaagcctggacacattttcattttccggggcgcggcagcacatacagcgattttaaatggcattggtaccattttgacggaaccgattgggacgagtcccgaaagctgaaccgcatctataagtttcaaggaaaggcttgggattgggaagtttccaatgaaaacggcaactatgattatttgatgtatgccgacatcgattatgaccatcctgatgtcgcagcagaaattaagagatggggcacttggtatgccaatgaactgcaattggacggtttccgtcttgatgctgtcaaacacattaaattttcttttttgcgggattgggttaatcatgtcagggaaaaaacggggaaggaaatgtttacggtagctgaatattggcagaatgacttgggcgcgctggaaaactatttgaacaaaacaaattttaatcattcagtgtttgacgtgccgcttcattatcagttccatgctgcatcgacacagggaggcggctatgatatgaggaaattgctgaacggtacggtcgtttccaagcatccgttgaaatcggttacatttgtcgataaccatgatacacagccggggcaatcgcttgagtcgactgtccaaacatggtttaagccgcttgcttacgcttttattctcacaagggaatctggataccctcaggttttctacggggatatgtacgggacgaaaggagactcccagcgcgaaattcctgccttgaaacacaaaattgaaccgatcttaaaagcgagaaaacagtatgcgtacggagcacagcatgattatttcgaccaccatgacattgtcggctggacaagggaaggcgacagctcggttgcaaattcaggtttggcggcattaataacagacggacccggtggggcaaagcgaatgtatgtcggccggcaaaacgccggtgagacatggcatgacattaccggaaaccgttcggagccggttgtcatcaattcggaaggctggggagagtttcacgtaaacggcgggtcggtttcaatttatgttcaaagatagacgcgtagggcccgcggctagcggccgcgtcgactagaagagcagagaggacggatttcctgaaggaaatccgtttttttattttgcccgtcttataaatttcgttgtccaactcgcttaattgcgagtttttatttcgtttatttcaatcaaggtaaatgctagcggccgcgtcgactagaagagcagagaggacggatttcctgaaggaaatccgtttttttattttgcccgtcttataaatttcgttgagatcttttatacaaataggcttaacaataaagtaaatcctaatccggccaccgcgataattgtttcaagcagtgtccaggtggcgaatgtttctttcatgctcaggccgaaatactctttgaacatccagaagcccgcgtcgttgacatgggaagcgattacacttccggcccctgttgcaagcacaaccagtgcaagattgacatcgctttgtccgagcatcggaagaacgagtccggtcgtgcttaatgcagcaactgtcgcggaacctaaagagatgcgcagaatcgcggcgatgacccaggcgagcaagatcggcgacatggccgttcctttgaataattcagctacatagtcgcctactccgccgttgatcaagacttgtttgaatgcgccgccgcccccgatgatcaagagcatcattccgatttgagtaatggcggttgaacaggaatccatcacttgtttgatcgggatctttctggcgatacccatcgtataaatcg

SEQ ID NO: 8 - DNA, 3594 bp, Artificial Sequence
  Sequence of the amyL locus after re-integration of amyL in PP3811-amyL3
tacagaagcatgaagggcatgcgaccttctttgtgcttggaagcagagcgcaatattatcccgaaacgataaaacggatgctgaaggaaggaaacgaagtcggcaaccattcctgggaccatccgttattgacaaggctgtcaaacgaaaaagcgtatcaggagattaacgacacgcaagaaatgatcgaaaaaatcagcggacacctgcctgtacacttgcgtcctccatacggcgggatcaatgattccgtccgctcgctttccaatctgaaggtttcattgtgggatgttgatccggaagattggaagtacaaaaataagcaaaagattgtcaatcatgtcatgagccatgcgggagacggaaaaatcgtcttaatgcacgatatttatgcaacgtccgcagatgctgctgaagagattattaaaaagctgaaagcaaaaggctatcaattggtaactgtatctcagcttgaagaagtgaagaagcagagaggctattgaataaatgagtagaaagcgccatatcggcgcttttcttttggaagaaaatatagggaaaatggtacttgttaaaaattcggaatatttatacaatatcatatgtatcacattgaaaggaggggcctgctgtccagactgtccgctgtgtaaaaaaaaggaataaaggggggttgacattattttactgatatgtataatataatttgtataagaaaatggaggggccctcgaaacgtaagatgaaaccttagataaaagtgctttttttgttgcaattgaagaattattaatgttaagcttaattaaagataatatctttgaattgtaacgcccctcaaaagtaagaactacaaaaaaagaatacgttatatagaaatatgtttgaaccttcttcagattacaaatatattcggacggactctacctcaaatgcttatctaactatagaatgacatacaagcacaaccttgaaaatttgaaaatataactaccaatgaacttgttcatgtgaattatcgctgtatttaattttctcaattcaatatataatatgccaatacattgttacaagtagaaattaagacacccttgatagccttactatacctaacatgatgtagtattaaatgaatatgtaaatatatttatgataagaagcgacttatttataatcattacatatttttctattggaatgattaagattccaatagaatagtgtataaattatttatcttgaaaggagggatgcctaaaaacgaagaacattaaaaacatatatttgcaccgtctaatggatttatgaaaaatcattttatcagtttgaaaattatgtattatggccacattgaaaggggaggagaatcatgaaacaacaaaaacggctttacgcccgattgctgacgctgttatttgcgctcatcttcttgctgcctcattctgcagcagcggcggcaaatcttaatgggacgctgatgcagtattttgaatggtacatgcccaatgacggccaacattggaggcgtttgcaaaacgactcggcatatttggctgaacacggtattactgccgtctggattcccccggcatataagggaacgagccaagcggatgtgggctacggtgcttacgacctttatgatttaggggagtttcatcaaaaagggacggttcggacaaagtacggcacaaaaggagagctgcaatctgcgatcaaaagtcttcattcccgcgacattaacgtttacggggatgtggtcatcaaccacaaaggcggcgctgatgcgaccgaagatgtaaccgcggttgaagtcgatcccgctgaccgcaaccgcgtaatttcaggagaacacctaattaaagcctggacacattttcattttccggggcgcggcagcacatacagcgattttaaatggcattggtaccattttgacggaaccgattgggacgagtcccgaaagctgaaccgcatctataagtttcaaggaaaggcttgggattgggaagtttccaatgaaaacggcaactatgattatttgatgtatgccgacatcgattatgaccatcctgatgtcgcagcagaaattaagagatggggcacttggtatgccaatgaactgcaattggacggtttccgtcttgatgctgtcaaacacattaaattttcttttttgcgggattgggttaatcatgtcagggaaaaaacggggaaggaaatgtttacggtagctgaatattggcagaatgacttgggcgcgctggaaaactatttgaacaaaacaaattttaatcattcagtgtttgacgtgccgcttcattatcagttccatgctgcatcgacacagggaggcggctatgatatgaggaaattgctgaacggtacggtcgtttccaagcatccgttgaaatcggttacatttgtcgataaccatgatacacagccggggcaatcgcttgagtcgactgtccaaacatggtttaagccgcttgcttacgcttttattctcacaagggaatctggataccctcaggttttctacggggatatgtacgggacgaaaggagactcccagcgcgaaattcctgccttgaaacacaaaattgaaccgatcttaaaagcgagaaaacagtatgcgtacggagcacagcatgattatttcgaccaccatgacattgtcggctggacaagggaaggcgacagctcggttgcaaattcaggtttggcggcattaataacagacggacccggtggggcaaagcgaatgtatgtcggccggcaaaacgccggtgagacatggcatgacattaccggaaaccgttcggagccggttgtcatcaattcggaaggctggggagagtttcacgtaaacggcgggtcggtttcaatttatgttcaaagatagacgcgtagggcccgcggctagcggccgcgtcgactagaagagcagagaggacggatttcctgaaggaaatccgtttttttattttgcccgtcttataaatttcgttgtccaactcgcttaattgcgagtttttatttcgtttatttcaatcaaggtaaatggctagcgcggccgcgtcgacaggcctctttgattacattttataattaattttaacaaagtgtcatcagccctcaggaaggacttgctgacagtttgaatcgcataggtaaggcggggatgaaatggcaacgttatctgatgtagcaaagaaagcaaatgtgtcgaaaatgacggtatcgcgggtgatcaatcatcctgagactgtgacggatgaattgaaaaagcttgttcattccgcaatgaaggagctcaattatataccgaactatgcagcaagagcgctcgttcaaaacagaacacaggtcgtcaagctgctcatactggaagaaatggatacaacagaaccttattatatgaatctgttaacgggaatcagccgcgagctggaccgtcatcattatgctttgcagcttgtcacaaggaaatctctcaatatcggccagtgcgacggcattattgcgacggggttgagaaaagccgattttgaagggctcatcaaggtttttgaaaagcctgtcgttgta

SEQ ID NO: 9 - DNA, 3852 bp, Artificial Sequence
  Sequence of the lacA2 locus after integration of amyL in PP3811-amyL3
tgttgattggctttggcctccagctttttataaatggattcaccgaagctggttaagtagatatagtggttgcggctgtcctcctcgcttctctttttatagaccatattttctttttcaaaccgcttcaggatccggctgacatagccccggtccaggccgagcgtatcttgaatcagtttggctgtacaatcggccgtattgtgaatttcaaataatatccgggtttccgtcaatgaaaaagggctgtcataaatatgttcattcagaaaaccgagcacatttgtatagaatcgattgaactttctgaattttaaagtgatagaatgattgatttctgtcatctcaaaacctctctccctgtaaatcgttgctttaatcaattataataaaatagttgatttagtcaagtgtatggaaatgaagttaaaaatgttaatgatagattatattttacaaataaagaaagataaattcaatcatacaggaaaattcatccagcggccgctcgctttccaatctgaaggtttcattgtgggatgttgatccggaagattggaagtacaaaaataagcaaaagattgtcaatcatgtcatgagccatgcgggagacggaaaaatcgtcttaatgcacgatatttatgcaacgtccgcagatgctgctgaagagattattaaaaagctgaaagcaaaaggctatcaattggtaactgtatctcagcttgaagaagtgaagaagcagagaggctattgaataaatgagtagaaagcgccatatcggcgcttttcttttggaagaaaatatagggaaaatggtacttgttaaaaattcggaatatttatacaatatcatatgtatcacattgaaaggaggggcctgctgtccagactgtccgctgtgtaaaaaaaaggaataaaggggggttgacattattttactgatatgtataatataatttgtataagaaaatggaggggccctcgaaacgtaagatgaaaccttagataaaagtgctttttttgttgcaattgaagaattattaatgttaagcttaattaaagataatatctttgaattgtaacgcccctcaaaagtaagaactacaaaaaaagaatacgttatatagaaatatgtttgaaccttcttcagattacaaatatattcggacggactctacctcaaatgcttatctaactatagaatgacatacaagcacaaccttgaaaatttgaaaatataactaccaatgaacttgttcatgtgaattatcgctgtatttaattttctcaattcaatatataatatgccaatacattgttacaagtagaaattaagacacccttgatagccttactatacctaacatgatgtagtattaaatgaatatgtaaatatatttatgataagaagcgacttatttataatcattacatatttttctattggaatgattaagattccaatagaatagtgtataaattatttatcttgaaaggagggatgcctaaaaacgaagaacattaaaaacatatatttgcaccgtctaatggatagaaaggaggtgatccagccgcaccttatgaaaaatcattttatcagtttgaaaattatgtattatggccacattgaaaggggaggagaatcatgaaacaacaaaaacggctttacgcccgattgctgacgctgttatttgcgctcatcttcttgctgcctcattctgcagcagcggcggcaaatcttaatgggacgctgatgcagtattttgaatggtacatgcccaatgacggccaacattggaggcgtttgcaaaacgactcggcatatttggctgaacacggtattactgccgtctggattcccccggcatataagggaacgagccaagcggatgtgggctacggtgcttacgacctttatgatttaggggagtttcatcaaaaagggacggttcggacaaagtacggcacaaaaggagagctgcaatctgcgatcaaaagtcttcattcccgcgacattaacgtttacggggatgtggtcatcaaccacaaaggcggcgctgatgcgaccgaagatgtaaccgcggttgaagtcgatcccgctgaccgcaaccgcgtaatttcaggagaacacctaattaaagcctggacacattttcattttccggggcgcggcagcacatacagcgattttaaatggcattggtaccattttgacggaaccgattgggacgagtcccgaaagctgaaccgcatctataagtttcaaggaaaggcttgggattgggaagtttccaatgaaaacggcaactatgattatttgatgtatgccgacatcgattatgaccatcctgatgtcgcagcagaaattaagagatggggcacttggtatgccaatgaactgcaattggacggtttccgtcttgatgctgtcaaacacattaaattttcttttttgcgggattgggttaatcatgtcagggaaaaaacggggaaggaaatgtttacggtagctgaatattggcagaatgacttgggcgcgctggaaaactatttgaacaaaacaaattttaatcattcagtgtttgacgtgccgcttcattatcagttccatgctgcatcgacacagggaggcggctatgatatgaggaaattgctgaacggtacggtcgtttccaagcatccgttgaaatcggttacatttgtcgataaccatgatacacagccggggcaatcgcttgagtcgactgtccaaacatggtttaagccgcttgcttacgcttttattctcacaagggaatctggataccctcaggttttctacggggatatgtacgggacgaaaggagactcccagcgcgaaattcctgccttgaaacacaaaattgaaccgatcttaaaagcgagaaaacagtatgcgtacggagcacagcatgattatttcgaccaccatgacattgtcggctggacaagggaaggcgacagctcggttgcaaattcaggtttggcggcattaataacagacggacccggtggggcaaagcgaatgtatgtcggccggcaaaacgccggtgagacatggcatgacattaccggaaaccgttcggagccggttgtcatcaattcggaaggctggggagagtttcacgtaaacggcgggtcggtttcaatttatgttcaaagatagacgcgtagggcccgcggctagcggccgcgtcgactagaagagcagagaggacggatttcctgaaggaaatccgtttttttattttgcccgtcttataaatttcgttgtccaactcgcttaattgcgagtttttatttcgtttatttcaatcaaggtaaatgctagcatcgattacaacccggatcaatggcttaaatatccggacgtattaaaagaagatatccgcctgatgaaactgtcccgctgcaatgtgatgtctgtcggcattttctcctgggtttcgctcgagcctgaagaaggaagatttacatttgactggctcgatcaggttcttgatactttcaaggaaaacggaatttatgcgtttttggctacaccgagcggtgccagaccggcttggatgtccaaaaagtatccagaggtgctgagaacggagcgcaacagggtcagaaaccttcacggaaagcggcacaatcactgctatacgtcgcctgtctaccgccggaaaacggcgatcataaacggaaagctcgcggagcgctatgcgcatcacccggccgtcatcggctggcacatttctaatgaatacggcggagaatgccattgtgaactttgccaagacaagttcagagagtggctgctggcgaaatacaaaacgctggaccgcc

SEQ ID NO: 10 - DNA, 9550 bp, Artificial Sequence
  Sequence of the plasmid pPPamyL-attP
gagctcgttattaatctgttcagcaatcgggcgcgattgctgaataaaagatacgagagacctctcttgtatcttttttattttgagtggttttgtccgttacactagaaaaccgaaagacaataaaaattttattcttgctgagtctggctttcggtaagctagacaaaacggacaaaataaaaattggcaagggtttaaaggtggagattttttgagtgatcttctcaaaaaatactacctgtcccttgctgatttttaaacgagcacgagagcaaaacccccctttgctgaggtggcagagggcaggtttttttgtttcttttttctcgtaaaaaaaagaaaggtcttaaaggttttatggttttggtcggcactgccgacagcctcgcagagcacacactttatgaatataaagtatagtgtgttatactttacttggaagtggttgccggaaagagcgaaaatgcctcacatttgtgccacctaaaaaggagcgatttacatatgagttatgcagtttgtagaatgcaaaaagtgaaatcagctggactaaaaggcagagctcggtaccagatctaaagataatatctttgaattgtaacccccctcaaaagtaagaactacaaaaaaagaatacgttatatagaaatatgtttgaaccttcttcagattacaaatatattcggacggactctacctcaaatgcttatctaactatagaatgacatacaagcacaaccttgaaaatttgaaaatataactaccaatgaacttgttcatgtgaattatcgctgtatttaattttctcaattcaatatataatatgccaatacattgttacaagtagaaattaagacacccttgatagccttactatacctaacatgatgtagtattaaatgaatatgtaaatatatttatgataagaagcgacttatttataatcattacatatttttctattggaatgattaagattccaatagaatagtgtataaattatttatcttgaaaggagggatgcctaaaaacgaagaacattaaaaacatatatttgcaccgtctaatggatagaaaggaggtgatccagccgcaccttatgaaaaatcattttatcagtttgaaaattatgtattatggccacattgaaaggggaggagaatcatgaaacaacaaaaacggctttacgcccgattgctgacgctgttatttgcgctcatcttcttgctgcctcattctgcagcagcggcggcaaatcttaatgggacgctgatgcagtattttgaatggtacatgcccaatgacggccaacattggaggcgtttgcaaaacgactcggcatatttggctgaacacggtattactgccgtctggattcccccggcatataagggaacgagccaagcggatgtgggctacggtgcttacgacctttatgatttaggggagtttcatcaaaaagggacggttcggacaaagtacggcacaaaaggagagctgcaatctgcgatcaaaagtcttcattcccgcgacattaacgtttacggggatgtggtcatcaaccacaaaggcggcgctgatgcgaccgaagatgtaaccgcggttgaagtcgatcccgctgaccgcaaccgcgtaatttcaggagaacacctaattaaagcctggacacattttcattttccggggcgcggcagcacatacagcgattttaaatggcattggtaccattttgacggaaccgattgggacgagtcccgaaagctgaaccgcatctataagtttcaaggaaaggcttgggattgggaagtttccaatgaaaacggcaactatgattatttgatgtatgccgacatcgattatgaccatcctgatgtcgcagcagaaattaagagatggggcacttggtatgccaatgaactgcaattggacggtttccgtcttgatgctgtcaaacacattaaattttcttttttgcgggattgggttaatcatgtcagggaaaaaacggggaaggaaatgtttacggtagctgaatattggcagaatgacttgggcgcgctggaaaactatttgaacaaaacaaattttaatcattcagtgtttgacgtgccgcttcattatcagttccatgctgcatcgacacagggaggcggctatgatatgaggaaattgctgaacggtacggtcgtttccaagcatccgttgaaatcggttacatttgtcgataaccatgatacacagccggggcaatcgcttgagtcgactgtccaaacatggtttaagccgcttgcttacgcttttattctcacaagggaatctggataccctcaggttttctacggggatatgtacgggacgaaaggagactcccagcgcgaaattcctgccttgaaacacaaaattgaaccgatcttaaaagcgagaaaacagtatgcgtacggagcacagcatgattatttcgaccaccatgacattgtcggctggacaagggaaggcgacagctcggttgcaaattcaggtttggcggcattaataacagacggacccggtggggcaaagcgaatgtatgtcggccggcaaaacgccggtgagacatggcatgacattaccggaaaccgttcggagccggttgtcatcaattcggaaggctggggagagtttcacgtaaacggcgggtcggtttcaatttatgttcaaagatagacgcgtagggcccgcggctagcggccgcgtcgactagaagagcagagaggacggatttcctgaaggaaatccgtttttttattttgcccgtcttataaatttcgttgtccaactcgcttaattgcgagtttttatttcgtttatttcaattaaggtaactaaagatcctctagagtcgattatgtcttttgcgcagtcggcttaaaccagttttcgctggtgcgaaaaaagagtgtcttgtgacacctaaattcaaaatctatcggtcagatttataccgatttgattttatatattcttgaataacatacgccgagttatcacataaaagcgggaaccaatcatcaaatttaaacttcattgcataatccattaaactcttaaattctacgattccttgttcatcaataaactcaatcatttctttaattaatttatatctatctgttgttgttttctttaataattcatcaacatctacaccgccataaactatcatatcttctttttgatatttaaatttattaggatcgtccatgtgaagcatatatctcacaagacctttcacacttcctgcaatctgcggaatagtcgcattcaattcttctgtaattatttttatctgttcataagatttattaccctcatacatcactagaatatgataatgctcttttttcatcctaccttctgtatcagtatccctatcatgtaatggagacactacaaattgaatgtgtaactcttttaaatactctaaccactcggcttttgctgattctggatataaaacaaatgtccaattacgtcctcttgaatttttcttgttttcagtttcttttattacattttcgctcatgatataataacggtgctaatacacttaacaaaatttagtcatagataggcagcatgccagtgctgtctatctttttttgtttaaaatgcaccgtattcctcctttgcatatttttttattagaataccggttgcatctgatttgctaatattatatttttctttgattctatttaatatctcattttcttctgttgtaagtcttaaagtaacagcaacttttttctcttcttttctatctacaaccatcactgtacctcccaacatctgtttttttcactttaacataaaaaacaaccttttaacattaaaaacccaatatttatttatttgtttggacaatggacaatggacacctaggggggaggtcgtagtacccccctatgttttctcccctaaataaccccaaaaatctaagaaaaaaagacctcaaaaaggtctttaattaacatctcaaatttcgcatttattccaatttcctttttgcgtgtgatgcgctgcgtccattaaaaatcctagagctttgaaaccgaaagttaatagctgtcgctactactttcgcttacgctctaagtatattttaaggactgtcacacgcaaaaagttttctcggcataaaagtacctctacatctctaaatcgtctgtacgctgtttctcacgctttctatcgaccttctggacattatcctgtacaacatccataaactgtcccacacgctcaaatttggaatcattaaagaatttctctttaagcctattaaaccctttctcaaacccagggaaattcgccctcgcagcacgatataaagtcactgtactagcttgaaatttctctgatacattcaactgctcattcaaactatcattctctcgctttaatttattaacctctttacttttttcgtgatacccctctttccatgtattcactacttctttcaaactctctctacgtttttttaattcttgattttctgtgtaatagtctgtgctcttaatattttcgtaatcatcaacaatccgttctgcagaagagattgtttcttgcaggcgttcaaattcatcagcagttaatatctttctaccagtctcttcacgtccagagaacaaacctgtacgctcattttcataatcaaagggtttcgtagacctcatatgctctattccactctgtaactgcttatttgccttctgtaactcatccttaacttcttgcagttcctgtttatgaaatacagtatctttcttgtactgatccatcgctttatgttctcgttctgtaacctctttggacgtgcctctttcaagttcataacctttctcattcacatactcattaaatctatcttgtaattgagtaaagtctttcttgttgcctaactgttcttttgcagacaatctcccgtcctctgttaaagggacaaaaccaaagtgcatatgtgggactctttcatccagatggacagtcgcatacagcatattttccttaccgtattcattttctagaaactccaagctatctttaaaaaatcgttctatttcttctccgcttaaatcatcaaagaaatctttatcacttgtaaccagtccgtccacatgtcgaattgcatctgaccgaattttacgtttccctgaataattctcatcaatcgtttcatcaattttatctttatactttatattttgtgcgttaatcaaatcataatttttatatgtttcctcatgatttatgtctttattattatagtttttattctctctttgattatgtctttgtatcccgtttgtattacttgatcctttaactctggcaaccctcaaaattgaatgagacatgctacacctccggataataaatatatataaacgtatatagatttcataaagtctaacacactagacttatttacttcgtaattaagtcgttaaaccgtgtgctctacgaccaaaactataaaacctttaagaactttctttttttacaagaaaaaagaaattagataaatctctcatatcttttattcaataatcgcatccgattgcagtataaatttaacgatcactcatcatgttcatatttatcagagctcgtgctataattatactaattttataaggaggaaaaaatatgggcatttttagtatttttgtaatcagcacagttcattatcaaccaaacaaaaaataagtggttataatgaatcgttaataagcaaaattcatataaccaaattaaagagggttataatgaacgagaaaaatataaaacacagtcaaaactttattacttcaaaacataatatagataaaataatgacaaatataagattaaatgaacatgataatatctttgaaatcggctcaggaaaaggccattttacccttgaattagtaaagaggtgtaatttcgtaactgccattgaaatagaccataaattatgcaaaactacagaaaataaacttgttgatcacgataatttccaagttttaaacaaggatatattgcagtttaaatttcctaaaaaccaatcctataaaatatatggtaatataccttataacataagtacggatataatacgcaaaattgtttttgatagtatagctaatgagatttatttaatcgtggaatacgggtttgctaaaagattattaaatacaaaacgctcattggcattacttttaatggcagaagttgatatttctatattaagtatggttccaagagaatattttcatcctaaacctaaagtgaatagctcacttatcagattaagtagaaaaaaatcaagaatatcacacaaagataaacaaaagtataattatttcgttatgaaatgggttaacaaagaatacaagaaaatatttacaaaaaatcaatttaacaattccttaaaacatgcaggaattgacgatttaaacaatattagctttgaacaattcttatctcttttcaatagctataaattatttaataagtaagttaagggatgcataaactgcatcccttaacttgtttttcgtgtgcctattttttgtgaatcgacctgcaggcatgcaagcttaagcgagttggaatttaaatatgatatctacattatcagcagtaacatcaacctttgatacaaggttgttgacgattttctttttattatcatatgatagttcattaatcggaattgagcccaactgagttttaactaactcaaaaacatcagtagagtcattaaatttattttcgctaatcttagctttaagcagctttttctcagcctgaagggaatcagtacgatctttcaactcatccatagtgataaaatcatttaggtacaaatcagagttcttttgtatttttttatcgatctgtgaaatttgctttttaaatgacgaagtatcaagaataggttggttgttgccattgataattttcaataaggagtcattattttcttgaaatccaatcaggttgtcaataacagtattttctaaattacttaaatcataagttcctgaatcacactttttattgtcattatatactgtaattccttttgtttttcgaggaaatctatttgcacagtgatatttcatagtgcggcttccatcttttcttttgtggccaagaacaatttttaaaggtgctccacagtaaccgcaccttgccatccctgacagcatatatttagcttggaaaggtctagggttgttatttctttcataagtctgctgttgtctttcttctagctctttttgaacttttaaataagtctcataagggataattggtttgtgcataccttcaaataggctgtccttaaatttgatataaccacagtaaactggattatcaagtgtttgtcttagggtacgataagaccacggtatatctttaccgatgtgtccagattcattgagtttatctcttaattttgtaagtgatattcctgataaataatcagtgaatatttgttcaactattgtagcttgtaaaggaacaatttctaatatacctgtctttctgttgtggtaatacccaaaagctgtcttagtccacatcatagacttaccagatttcgctcgccctagtttacccatagtcatgcgttcttttatattctctctttcaaactcattaattgcagaaagaatagtgagaaacaagctacccatagcagaagaagtatcaatactttcattaagcgagataaagtctattttattttttgtgaacacatccttaacaagataaagagtatctcttacactacgtgaaaggcggtctagcttatatacaagaactgtatcaaaagctttattctcgatatcgttgattaatctttgcattgctgggcgttcaagtttggcccctgaaaaaccagcatcagtataagtatcagatacttgccaccccattgcttcagcatattttgttaaacggtcaatttgctcatcaattgagaacccttcctctgcttggttagtagtggatactcgtgtatagattgctactttcttagtcatgagatttcccccttaaaaataaattcattcaaatacagatgcattttatttcatatagtaagtacatcacctattagtttgttgtttaaacaaactaacttattttcatcttatataacctcgtcagtattttcaatattttttttagttttttatgaacacattagatttaataaagggaagattcgctatgtactatgttgatacttaatttaaagattaaacaaatggagtggatgaagtggatatcgctgatcaaacctttgtcaaaaaagtaaatcaaaagttattattaaaagaaatccttaaaaattcacctatttcaagagcaaaattatctgaaatgactggattaaataaatcaactgtctcatcacaggtaaacacgttaatgaaagaaagtatggtatttgaaataggtcaaggacaatcaagtggcggaagaagacctgtcatgcttgtttttaataaaaaggcaggatactccgttggaatagatgttggtgtggattatattaatggcattttaacagaccttgaaggaacaatcgttcttgatcaataccgccatttggaatccaattctccagaaataacgaaagacattttgattgatatgattcatcactttattacgcaaatgccccaatctccgtacgggtttattggtataggtatttgcgtgcctggactcattgataaagatcaaaaaattgttttcactccgaactccaactggagagatattgacttaaaatcttcgatacaagagaagtacaatgtgtctgtttttattgaaaatgaggcaaatgctggcgcatatggagaaaaactatttggagctgcaaaaaatcacgataacattatttacgtaagtatcagcacaggaatagggatcggtgttattatcaacaatcatttatatagaggagtaagcggcttctctggagaaatgggacatatgacaatagactttaatggtcctaaatgcagttgcggaaaccgaggatgctgggaattgtatgcttcagagaaggctttattaaaatctcttcagaccaaagagaaaaaactgtcctatcaagatatcataaacctcgcccatctgaatgatatcggaaccttaaatgcattacaaaattttggattctatttaggaataggccttaccaatattctaaatactttcaacccacaagccgtaattttaagaaatagcataattgaatcgcatcctatggttttaaattcaatgagaagtgaagtatcatcaagggtttattcccaattaggcaatagctatgaattattgccatcttccttaggacagaatgcaccggcattaggaatgtcctccattgtgattgatcattttctggacatgattacaatgtaattttttatggaatggacagctcatctttaaagatgagtttttttattctaggagtatttctgaattc

SEQ ID NO: 11 - DNA, 22 bp, Artificial Sequence
  Primer 1
gtttcacgtaaacggcgggtcg

SEQ ID NO: 12 - DNA, 23 bp, Artificial Sequence
  Primer 2
gatgggtatcgccagaaagatcc

SEQ ID NO: 13 - DNA, 23 bp, Artificial Sequence
  Primer 3
caacgacaggcttttcaaaaacc

SEQ ID NO: 14 - DNA, 23 bp, Artificial Sequence
  Primer 4
cggtccagcgttttgtatttcgc

SEQ ID NO: 15 - DNA, 1612 bp, Artificial Sequence
  Sequence of BgIII-MluI fragment
agatctgtaaagataatatctttgaattgtaacccccctcaaaagtaagaactacaaaaaaagaatacgttatatagaaatatgtttgaaccttcttcagattacaaatatattcggacggactctacctcaaatgcttatctaactatagaatgacatacaagcacaaccttgaaaatttgaaaatataactaccaatgaacttgttcatgtgaattatcgctgtatttaattttctcaattcaatatataatatgccaatacattgttacaagtagaaattaagacacccttgatagccttactatacctaacatgatgtagtattaaatgaatatgtaaatatatttatgataagaagcgacttatttataatcattacatatttttctattggaatgattaagattccaatagaatagtgtataaattatttatcttgaaaggagggatgcctaaaaacgaagaacattaaaaacatatatttgcaccgtctaatggatagaaaggaggtgatccagccgcaccttatgaaaaatcattttatcagtttgaaaattatgtattatgtggccagaagttcctattccgaagttcctattctctagaaagtataggaacttcttataaaaatgaggagggaaccgaatgagtaaaggagaagaacttttcactggagttgtcccaattcttgttgaattagatggcgatgttaatgggcaaaaattctctgttagtggagagggtgaaggtgatgcaacatacggaaaacttacccttaaatttatttgcactactgggaagctacctgttccatggccaacgcttgtcactactctcacttatggtgttcaatgcttttctagatacccagatcatatgaaacagcatgactttttcaagagtgccatgcccgaaggttatgtacaggaaagaactatattttacaaagatgacgggaactacaagacacgtgctgaagtcaagtttgaaggtgatacccttgttaatagaatcgagttaaaaggtattgattttaaagaagatggaaacattcttggacacaaaatggaatacaattataactcacataatgtatacatcatggcagacaaaccaaagaatggcatcaaagttaacttcaaaattagacacaacattaaagatggaagcgttcaattagcagaccattatcaacaaaatactccaattggcgatggccctgtccttttaccagacaaccattacctgtccacgcaatctgccctttccaaagatcccaacgaaaagagagatcacatgatccttcttgagtttgtaacagctgctgggattacacatggcatggatgaactatacaaataatgctgtccagactgtccgctgtgtaaaaaaaaggaataaaggggggttgacattattttactgatatgtataatataatttgtataagaaaatgcttcatgtaatggtcaaaatgttttagagctagaaatagcaagttaaaataaggctagtccgttatcaacttgaaaaagtggcaccgagtcggtgctttgaagttcctattccgaagttcctattcttcaaatagtataggaacttcacgcgt